European Patent Application EP 4 424 822 A1, published September 4, 2024. Title: Designer recombinase for the precise excision of HTLV-1 provirus. Applicant: PROVIREX Genome Editing Therapies GmbH. The sequence listing filed with the application follows.

SEQUENCE LISTING (39 sequences)

SEQ ID NO: 1 - DNA, 34 bp, HTLV-1
  source 1..34: mol_type = other DNA; note = loxHTLV-1
acaggagtctataaaagcgtggagacagttcagg

SEQ ID NO: 2 - DNA, 34 bp, synthetic construct
  source 1..34: mol_type = other DNA; note = subsite 1
acaggagtctataaaagcgtgtatagcatcctgt

SEQ ID NO: 3 - DNA, 34 bp, synthetic construct
  source 1..34: mol_type = other DNA; note = subsite 1A
acaggattctataaaagcgtgtatagcatcctgt

SEQ ID NO: 4 - DNA, 34 bp, unidentified
  source 1..34: mol_type = other DNA; note = subsite 1B
acaacagtctataaaagcgtgtatagcatgttgt

SEQ ID NO: 5 - DNA, 34 bp, synthetic construct
  source 1..34: mol_type = other DNA; note = subsite 2
acaacattgtataaaagcgtggagacagttcagg

SEQ ID NO: 6 - DNA, 34 bp, synthetic construct
  source 1..34: mol_type = other DNA; note = subsite 2A
acaacattgtataaaagcgtgtagacagtgctgg

SEQ ID NO: 7 - DNA, 34 bp, synthetic construct
  source 1..34: mol_type = other DNA; note = subsite 2B
acaacatcgtataaaagcgtggataccattcagg

SEQ ID NO: 8 - DNA, 34 bp, synthetic construct
  source 1..34: mol_type = other DNA; note = subsite 2C
acaacattgtataaaagcgtggagaccatgctgg

SEQ ID NO: 9 - DNA, 34 bp, bacteriophage P1
  source 1..34: mol_type = other DNA; note = loxP
ataacttcgtataatgtatgctatacgaagttat

SEQ ID NO: 10 - DNA, 92 bp, Homo sapiens
  source 1..92: mol_type = genomic DNA
caaacatccacttggtgttttccattagtgttataccgttattgtttgcataatgacagggatacctctgaggaatatgtctttaggcaatt

SEQ ID NO: 11 - protein, 343 aa, bacteriophage P1
  source 1..343: note = Cre
MSNLLTVHQNLPALPVDATSDEVRKNLMDMFRDRQAFSEHTWKMLLSVCRSWAAWCKLNNRKWFPAEPEDVRDYLLYLQARGLAVKTIQQHLGQLNMLHRRSGLPRPSDSNAVSLVMRRIRKENVDAGERAKQALAFERTDFDQVRSLMENSDRCQDIRNLAFLGIAYNTLLRIAEIARIRVKDISRTDGGRMLIHIGRTKTLVSTAGVEKALSLGVTKLVERWISVSGVADDPNNYLFCRVRKNGVAAPSATSQLSTRALEGIFEATHRLIYGAKDDSGQRYLAWSGHSARVGAARDMARAGVSIPEIMQAGGWTNVNIVMNYIRNLDSETGAMVRLLEDGD

SEQ ID NO: 12 - protein, 343 aa, synthetic construct
  source 1..343: note = consensus sequence of E5 and G9
MSKLLTXXQDLSALLADXTSDEARKNLMDMFRDRQAFPEHTWXMLLSVCRSWAAWCESNNRKWFPAEPEDVRDYLLHLQARGLTVNTVQKHLAELNTLHRRSGLPRPGDXNAVXLVMRRIRRENVDAGERAKQALAFERTDFDXVRXLMENSDRXXDIRNLAFLGVAYNTLLRISEIARIRVXDISRTDGGRMLIHIGRTKTLVSXAGVEKALSLGVTKLVERWIXXSGVADDPNNYLFCRVRRYGVVVXSATSRLSTHAMQGIFGXAHRLIYGAKDDSGQRYLAWSGHSARVGAARDXARAGVSIAEIMQAGGWTRVXSVMNYIRNLDSETGAMVRLLEDGX

SEQ ID NO: 13 - protein, 343 aa, synthetic construct
  source 1..343: note = G9
MSKLLTLHQDLSALLADVTSDEARKNLMDMFRDRQAFPEHTWEMLLSVCRSWAAWCESNNRKWFPAEPEDVRDYLLHLQARGLTVNTVQKHLAELNTLHRRSGLPRPGDSNAVTLVMRRIRRENVDAGERAKQALAFERTDFDRVRSLMENSDRCLDIRNLAFLGVAYNTLLRISEIARIRVKDISRTDGGRMLIHIGRTKTLVSAAGVEKALSLGVTKLVERWITASGVADDPNNYLFCRVRRYGVVVSSATSRLSTHAMQGIFGTAHRLIYGAKDDSGQRYLAWSGHSARVGAARDLARAGVSIAEIMQAGGWTRVNSVMNYIRNLDSETGAMVRLLEDGD

SEQ ID NO: 14 - protein, 343 aa, synthetic construct
  source 1..343: note = E5
MSKLLTIYQDLSALLADATSDEARKNLMDMFRDRQAFPEHTWKMLLSVCRSWAAWCESNNRKWFPAEPEDVRDYLLHLQARGLTVNTVQKHLAELNTLHRRSGLPRPGDNNAVSLVMRRIRRENVDAGERAKQALAFERTDFDQVRALMENSDRRQDIRNLAFLGVAYNTLLRISEIARIRVRDISRTDGGRMLIHIGRTKTLVSTAGVEKALSLGVTKLVERWISVSGVADDPNNYLFCRVRRYGVVVPSATSRLSTHAMQGIFGAAHRLIYGAKDDSGQRYLAWSGHSARVGAARDMARAGVSIAEIMQAGGWTRVDSVMNYIRNLDSETGAMVRLLEDGY

SEQ ID NO: 15 - protein, 343 aa, synthetic construct
  source 1..343: note = Tre
MSNLLTLHHSLPALPADATSDEVRKNLMDVFRDRPAFSEHTWEMLLSVCRSWAAWCKLNNRKWFPAEPEDVRDYLLHLQARGLAVKTIQQHLCRLNMLHRRSGLPRPSDSNAVSLVMRRIRKENVDAGERTKQALAFERTDFDQVRSLMENSDRCQDIRNLAFLGVAYNTLLRIAEIARIRVKDISRTDGGRMLIHIGRTKTLVSTAGVEKALSLGVTKLVERWISVSGVADDPNNYLFCRVRRYGVAAPSATSQLSTYALQRIFEATHRLIYGAKDDSGQRYLAWSGHSARVGAARDMARAGVSIPEIMQAGGWTTVNSVMNYIRNLDSETGAMVRLLEDGD

SEQ ID NO: 16 - protein, 343 aa, synthetic construct
  source 1..343: note = Brec1
MSILLTLHQSLSALLVDATSDEARKNLMDVLRDRQAFSERTWKVLLSVCRTWAAWCKLNNRKWFPAEPEDVRDYLLHLQARGLAVNTILQHLAQLNMLHRRFGLPRPGDSDAVSLVMRRIRRENVDAGERTKQALAFERTDFDQVRALMENSERGQDIRTLALLGVAYNTLLRVSEIARIRIKDISRTDGGRMLIHISRTKTLVSTAGVEKALSLGVTKLVERWISVSGVASDPNNYLFCQVRINGVAVPSATSRLSTDVLRKIFEAAHRLIYGAKDGSGQRYLAWSGHSARVGAARDMARAGVSIAEIMQAGGWTTVESVMNYIRNLDSETGAMVRLLEDGD

SEQ ID NO: 17 - DNA, 34 bp, Homo sapiens
  source 1..34: mol_type = genomic DNA
acagtcgtctttaccttgggggagacagttgtgg

SEQ ID NO: 18 - DNA, 34 bp, Homo sapiens
  source 1..34: mol_type = genomic DNA
ccagaagtctatcaggacagagagattgtccagg

SEQ ID NO: 19 - DNA, 34 bp, Homo sapiens
  source 1..34: mol_type = genomic DNA
acagcagtctgaagttgacctgagacacttgagc

SEQ ID NO: 20 - DNA, 34 bp, Homo sapiens
  source 1..34: mol_type = genomic DNA
acagcagtctgaagttgacctgagacatttgagc

SEQ ID NO: 21 - DNA, 34 bp, Human immunodeficiency virus 1
  source 1..34: mol_type = other DNA; note = loxLTR
acaacatcctattacaccctatatgccaacatgg

SEQ ID NO: 22 - DNA, 34 bp, Human immunodeficiency virus 1
  source 1..34: mol_type = other DNA; note = loxBTR
aacccactgcttaagcctcaataaagcttgcctt

SEQ ID NO: 23 - DNA, 34 bp, Homo sapiens
  source 1..34: mol_type = genomic DNA
tattgtttgcataatgacagggatacctctgagg

SEQ ID NO: 24 - protein, 343 aa, synthetic construct
  source 1..343: note = Library of recombinases
MSNLQTLHQSLSALLVDATSDEARQNLMVTFRDHQAFPEHTWKMLLSVCRSWAAWCELNNRKWFPAEPEDVRDYLLHLQARGLTVNTIQKHLAELNTLHRRSGLPRPGDSNAVSLVMRRIRRENVDAGERAKQALAFERTDFDQVRSLMENSDRCQDIRNLAFLGVAYNTLLRISEIARIRVKDISRTDGGRMLIHIGRTKTLVSTAGVEKALSLGVTKLVERWISVSGVADDPNNYLFCRVRRYGVVVPSATSQLSTHAMQGIFGAAHRLIYGAKDDSGQRYLAWSGHSARVGAARDMARAGVSIAEIMQAGGWTTVNSVMNYIRNLDSETGAMVRLLEDGD

SEQ ID NO: 25 - protein, 7 aa, synthetic construct
  source 1..7: note = Nuclear localization signal
PKKKRKV

SEQ ID NO: 26 - protein, 343 aa, synthetic construct
  source 1..343: note = A3_A9_C6
MSDLQTLHQDLSALLADVTSDEARQNLMVTFRDHQAFPEHTWKMLLSVCRSWAAWCELDNRKWFPAEPEDVRDYLLYLQARGLTVSTIQKHLAELNTLHRRSGLPRPGDSNAVSLVMRRIRRENVDAGERAKQALAFERTDFDQVRPLMESSDRRQDIRNLAFLGVAYNTLLRISEIARIRVKDISRTDGGRMLIHIGRTKTLVSTAGVEKALSLGVTKLVERWISVSGVADDPNNYLFCRVRRYGVVVPSATSRLSTHAMQGIFGAAHRLIYGAKDDSGQRYLAWSGHSARVGAARDMARAGVSIPEIMQAGGWTTVNSVMNYIRNLDSETGAMVRLLEDGD

SEQ ID NO: 27 - protein, 343 aa, synthetic construct
  source 1..343: note = A11_E1
MSNLQTLHQDLSALLVDATSDEARRNLMVTLRDHQAFPEHTWKMLLSVCRSWAAWCELNNRKWFPAEPEDVRDYLLHLQARGLTVNTIQKHLAELNTLHRRSGLPRPGDSNAVSLVMRRIRRENVDAGERAKQALAFERTDFDRVRSLMENSDRCQDIRNLAFLGVAYNTLLRISEIARIRVKDISRTDGGRMLIHIGRTKTLVSTAGVEKALSLGVTKLVERWISVSGVADDPDNYLFCRVRRYGVVAPSAANRLSTHAMQGIFGAAHRLIYGAKDDSGQRYLAWSGHSARVGAARDMARAGVSIAEIMQAGGWTRVDTVMNYIRNLDSETGAMVRLLEDGD

SEQ ID NO: 28 - protein, 343 aa, synthetic construct
  source 1..343: note = B12
MSKLQTLHQNLSALLADAMSDEARKSLTITLRDCQAFPEHTWKMLLSVCRSWAAWCELNNRKWFPAEPEDVRDYLLYLQARGLTVNTIQKHLAELNTLHRRSGLPRPGDSSAVSLVMRRIRRENIDAGERAKQALAFERADFDRVRSLMENSDRRQDIRNLAFLGVAYNTLLRISEIARIRVKDISRTDGGRMLIHIGRTKTLVSTAGVEKALSLGVTKLVERWISVSGVANDPDNYLFCRVRRYGVVVPSATSRLSTHAMQGIFGAAHRLIYGAKDDSGQRYLAWSGHSARVGAARDMARAGVSMAEIMQAGGWTRVDTVMNYIRNLDSETGAMVRLLEDGD

SEQ ID NO: 29 - protein, 343 aa, synthetic construct
  source 1..343: note = C2
MSNLQTLHHSLSALLVDATSDEARQNLMVTLRDHQAFPEHTWKMLLSVCRSWAAWCKLNNRRWFPAEPEDVRDYLLHLQARGLTVNTIQKHLAELNTLHRRSGLPRPGDSNAVSLVMRRIRRENVDAGERAKQALAFERTDFDQVRSLMENSDRRQDIRNLAFLGVAYNTLLRISEIARIRVKDISRTDGGRMLIRIGRTKTLVSTAGVEKALSLGVTKLVERWISVSGVADDPNNYLFCRVRKYGIAAPSATSQLSTHAMQGIFGAAHRLIYGAKDDSGQRYLAWSGHSARVGAARDMARAGVSIVEIMQAGGWTRVDTVMNYIRNLDSETGAMVRLLEGDD

SEQ ID NO: 30 - protein, 343 aa, synthetic construct
  source 1..343: note = D7
MSKLQTLPHSLSALLVDATSDEARRNLMVTFRDHQAFPEHTWKMLLSVCRTWAAWCELNNRKWFPAEPEDVRDYLLYLQARGLTVNTIQKHLTELNTLHRRSGLPRPGDSNAVPLVMRRIRRENVDAGERAKQALAFERTDFDRVRSLMENSDRCQDIRNLAFLGVAYNTLLRISEIARIRVRDISRTDGGRMLIHIGRTKTLVSTAGVEKALSLGVTRLVERWISVSGVADDPNNYLFCQVRKYGIAAPSATCQLSTGALRKIFGTAHRLIYGAKDDSGRRYLAWSGHSARVGAARDMARAGVSIPEIMQAGGWTTVNGVMNYIRNLDSETGAMVRLLEDGD

SEQ ID NO: 31 - protein, 343 aa, synthetic construct
  source 1..343: note = D11_F7_F9_G8
MSNLPTLHQNLSALLVGVTSDEARKNLMVMFRDRQAFPEHTWKMFLSVCRSWAAWCELNNRKWFPAEPEDVRDYLLHLQARGLTVNTVQKHLAELNTLHRRSGLPRPGDSNAVSLVMRRIRRENVDAGERAKQALAFERTDFDQVRSLMENSDRCQDIRNLAFLGVAYNTLLRISEIARIRVKDISRTDGGRMLIHIGRTKTLVSTAGVEKALSLGVTKLVERWISVSGVTDDPNNYLFCRVRKYGIAAPSATSQLSTGALRKVFGAAHRLVYGARDGSSQRYLAWSGHSARVGAARDMARAGASMAEIMQAGGWTRVDTVMNYIRNLDSETGAMVRLLEDGD

SEQ ID NO: 32 - protein, 343 aa, synthetic construct
  source 1..343: note = F6
MSNLQTLHHSLSALLADVASDEARKNLMDMFRDRQAFPEHTWKMFLSVCRSWAAWCKLNNRKWFPAEPEDVRDYLLHLQARGLTVNTVQKHLAELNMLHRRSGLPRPGDSNAVSLVMRRIRRENVDAGERAKQALAFERTDFDQVRTLMENSDRRKDIRDLAFLGVAYNTLLRISEIARIRVRDISRTDGGRMLIHIGRTKTLVSTAGVEKALSLGVTKLIERWISVSGVADDPNNYLFCRVRRYGVVVPSATSRLSTHAMQGIFGAAHRLIYGAKDDSGQRYLAWSGHSARVGAARDMARAGVSMAEIMQAGGWTRVDTVMNYIRNLDSEAGAMVRLLEDGD

SEQ ID NO: 33 - protein, 343 aa, synthetic construct
  source 1..343: note = F11
MSNLQTLHQDLSALLADAMSDEARRSLMVVLRDHQAFPEHTWKMLLSVCRAWAAWCELNNRKWFPAEHEDVRDYLLHLQARGLTVSTIQKHLAELNTLHRRSGLPRPGDSNAVSLVMRRIRRENVDAGERAKQALAFERTDFDRVRSLMETSDRRQDIRNLAFLGVAYNTLLRISEIARIRVKDISRTDGGRMLIHIGRTKTLVSTTGVEKALSLGVTKLVERWISVSCVADDPNNYLFCRVRRYGVVVPSATSRLSTHAMQGIFGAAHRLIYGAKDDSGQRYLAWSGHSARVGAARDMARAGVSIAEIMQAGGWTTVNSVMNYIRNLDSETGAMVRLLEDGD

SEQ ID NO: 34 - protein, 343 aa, synthetic construct
  source 1..343: note = F12
MSNLQTLHQSLTALLVDATSDEARQNLMVTFRDHQAFPAHTWKMLLSVCRSWAAWCELNNRKRFPAEPEDVRDYLLYLQARGLTVNTVQKHLTDLNTLHRRSGLPRPGDSNAVSLVMRRIRRENVDAGERARQALAFERTDFDLVRSLMEDSDRCQDIRNLAFLGVAYNTLLRISEIARIRVKDVSRTDGGRMLIHIGRTKTLVSTAGVEKALSLGVTXLVERWISVSGVADDPNNYLFCRVRRYGVVVPSATKQLSAYAMQGIFGAAHRLIYGAKDDSGRRYLAWSGHSARVGAARDMARAGVSLPEIMQAGGWTRVDTVMNYIRNLDSETGAMVRLLEDGD

SEQ ID NO: 35 - protein, 343 aa, synthetic construct
  source 1..343: note = G7
MSNLLTLHHSLSASLVDATSDEARQNLMVTFRDHQAFPEHTWRMLLSVCRSWAAWCELNNRKWFPAEPEDVRDYLLYLQARGLTVNTIQKHLAELNTLHRRSGLPRPGDSNAVSLVMRRIRRENVDAGERAKQALAFERTDFDQVRSLMENSDCRQDIRNLAFLGVAYNTLLRISEIARIRVKDISRTDGGRMLIHIGRTKTLVSTAGVEKALSLGVTRLVERWVSVSGIADDPNNYLFCRVRRYGVVVPSATSRLSTHAMQGIFGAAHRLIYGAKDDSGQRYLAWSGHSARVGAARDMARAGVSIAEIMQAGGWTTVNSVMNYIRNLDSETGAMVRLLEDGD

SEQ ID NO: 36 - protein, 343 aa, synthetic construct
  source 1..343: note = G10
MSNLQTLHHSLSALLVNATSDEARKSLTIMLRDHQAFPEHTWKMLLSVCRSWAAWCELNNRKWFPAEPEDVRDYLLYLQARGLTVNTIQKHLAELNTLHRRSGLPRPGDSNAVSLVMRRIRRENVDAGERAKQALAFERTDFDRVRTLMENSDRRQDIRNLAFLGVAYNTLLRISEIARIRVKDISRTDGGRMLIHIGRTKTLVSTAGVEKALSLGVTKLVERWISVSGVADDPNNYLFCRVRRYGIAVPSATSRLSTHAMQGIFGAAHRLIYGAKGDSGLRYLAWSGHSARVGAARDMARAGVSIPEIMQAGGWTTVNSVMNYIRNLDSETGAMVRLLEDDD

SEQ ID NO: 37 - protein, 343 aa, synthetic construct
  source 1..343: note = H2
MSNLQTLHQNLSALLVDATSDEARQNLMVMFRDRHAFPEHTWEMLLSVCRSWAAWCELNNRKWFPAEPEDVRDYLLHLQARGLTVNTVQKHLAELNMLHRRSGLPRPGDSNAVSLVMRRIRRENVDAGERAKQALPFERTDFDQVRSLLENSDRRLDIRNLAFLGVAYNTLLRISEIARIRVKDISRTDGGRMLIRIGRTKTLVSTAGVEKALSLGVTKLVERWFSVSGVADDPNNYLFCRVRRYGVVVPSATSQLSAYAMQGIFGAAHRLIYGANDDSGRRYLAWSGHSARVGAARDMARAGVSLPEIMQAGGWTTVNSVMNYIRNLDSETGAMVRLLEEGD

SEQ ID NO: 38 - protein, 343 aa, synthetic construct
  source 1..343: note = consensus sequence of all clones
MSXLXTXXXXLXAXLXXXXSDEXRXXLXXXXRDXXAFPXHTWXMXLSVCRXWAXWCXXXNRXXFPAEXEDVRDYLLXLQARGLTVXTXQKHLXXLNXLHRRSGLPRPGDXXAVXLVMRRIRRENXDAGERAXQALXFERXDFDXVRXLXEXSDXXXDIRXLAFLGVAYNTLLRISEIARIRVXDXSRTDGGRMLIXIGRTKTLVSXXGVEKALSLGVTXLXERWXXXSXXXXDPXNYLFCXVRXYGXXXXSAXXXLSXXAXXXXFGXAHRLXYGAXXXSXXRYLAWSGHSARVGAARDXARAGXXXXEIMQAGGWTXVXXVMNYIRNLDSEXGAMVRLLEXXX

SEQ ID NO: 39 - protein, 343 aa, synthetic construct
  source 1..343: note = B11
MSNLLTLHQDLFALLVDATSDETRRNLMDMFRDRQAFPEHTWKMLLSVCRSWATWCELNNRKWFPAEPEDVRDYLLDLQARGLTVNTIQKHLAELNMLHRRSGLPRPGDSSAVSLVMRRIRRENVDAGERAKQALAFERTDFDQVRSLMENSDRRQDIRNLAFLGVAYNTLLRISEIARIRVKDISRTDGGRMLIHIGRTKTLVSTAGVEKALSLGVTKLVERWISVSGVADDPNNYLFCRVRKYGIAAPSATSQLSTGALRKIFGAAHRLIYGAKDDSGQRYLAWSGHSARVGAARDMARAGVPIAEIMQAGGWTRVDTVMNYIRNLDSETGAMVRLLEDGD